European Patent Specification EP 3 400 309 B1, published March 19, 2025. Title: METHODS AND COMPOSITIONS FOR DETECTING CANDIDA SPECIES. Applicant: Gen-Probe Incorporated JIANG, Alice GETMAN, Damon HUDSON, Angela EATON, Barbara. The sequence listing filed with the application follows.

SEQUENCE LISTING (155 sequences)

SEQ ID NO: 1-2 - skipped (2 entries)

SEQ ID NO: 3 - DNA, 25 bp, Artificial Sequence
  Synthetic Oligonucleotide
ccaaguccuuguggcuuggccuugg

SEQ ID NO: 4 - DNA, 28 bp, Artificial Sequence
  Synthetic Oligomer
augggaauggcgccguggauggucccau

SEQ ID NO: 5 - skipped

SEQ ID NO: 6 - DNA, 18 bp, Artificial Sequence
  Synthetic Oligomer
gtgggaaattcggtggta

SEQ ID NO: 7 - DNA, 22 bp, Artificial Sequence
  Synthetic Oligomer
gaaattcggtggtacgctccat

SEQ ID NO: 8 - skipped

SEQ ID NO: 9 - DNA, 46 bp, Artificial Sequence
  Synthetic Oligonucleotide
  promoter (1)..(27)
aatttaatacgactcactatagggagatcaagttcgcatattgcac

SEQ ID NO: 10 - DNA, 47 bp, Artificial Sequence
  Synthetic oligomer
  promoter (1)..(27)
aatttaatacgactcactatagggagatgatcggtatcgggtgcttg

SEQ ID NO: 11 - DNA, 19 bp, Artificial Sequence
  Synthetic Oligonucleotide
agtgcattggagtttctgc

SEQ ID NO: 12 - DNA, 18 bp, Artificial Sequence
  Synthetic Oligonucleotide
gcattggagtttctgctg

SEQ ID NO: 13 - DNA, 45 bp, Artificial Sequence
  Synthetic Oligonucleotide
  promoter (1)..(27)
aatttaatacgactcactatagggagaaccgacatccttacgtag

SEQ ID NO: 14 - DNA, 49 bp, Artificial Sequence
  Synthetic Oligonucleotide
  promoter (1)..(27)
aatttaatacgactcactatagggagaatactggaccgacatccttacg

SEQ ID NO: 15-17 - skipped (3 entries)

SEQ ID NO: 18 - DNA, 22 bp, Artificial Sequence
  Synthetic Oligonucleotide
gguggauuugugcgacaccacc

SEQ ID NO: 19 - DNA, 27 bp, Artificial Sequence
  Synthetic Oligonucleotide
augggaauggcgccguggauggcccau

SEQ ID NO: 20 - skipped

SEQ ID NO: 21 - DNA, 25 bp, Artificial Sequence
  Synthetic Oligonucleotide
ggcagagacguaugggccugcugcc

SEQ ID NO: 22 - skipped

SEQ ID NO: 23 - DNA, 52 bp, Artificial Sequence
  Synthetic Oligonucleotide
  misc_feature (20)..(52): 3' Tail
tcggtatcgggtgcttgaatttaaaaaaaaaaaaaaaaaaaaaaaaaaaaaa

SEQ ID NO: 24 - DNA, 53 bp, Artificial Sequence
  Synthetic Oligonucleotide
  misc_feature (21)..(53): 3' Tail
agatcggtatcgggtgcttgtttaaaaaaaaaaaaaaaaaaaaaaaaaaaaaa

SEQ ID NO: 25 - skipped

SEQ ID NO: 26 - DNA, 21 bp, Artificial Sequence
  Synthetic Oligonucleotide
cgttacaagaaatatacacgg

SEQ ID NO: 27 - DNA, 28 bp, Artificial Sequence
  Synthetic Oligonucleotide
ggaauggcgccguggaugguugcauugg

SEQ ID NO: 28 - DNA, 23 bp, Artificial Sequence
  Synthetic Oligonucleotide
gccgucagccaaccauccacggc

SEQ ID NO: 29-30 - skipped (2 entries)

SEQ ID NO: 31 - DNA, 17 bp, Artificial Sequence
  Synthetic Oligonucleotide
ggcgttacaagaaatat

SEQ ID NO: 32 - DNA, 19 bp, Artificial Sequence
  Synthetic Oligonucleotide
gcggcgttacaagaaatat

SEQ ID NO: 33 - skipped

SEQ ID NO: 34 - DNA, 21 bp, Artificial Sequence
  Synthetic Oligonucleotide
ggtagtttggcttttctttgg

SEQ ID NO: 35 - skipped

SEQ ID NO: 36 - DNA, 58 bp, Artificial Sequence
  Synthetic Oligonucleotide
  misc_feature (26)..(58): 3' Tail
ggatggagcgtaccaccgaatttcctttaaaaaaaaaaaaaaaaaaaaaaaaaaaaaa

SEQ ID NO: 37 - DNA, 53 bp, Artificial Sequence
  Synthetic Oligonucleotide
  misc_feature (21)..(53): 3' Tail
taccaccgaatttcccaccctttaaaaaaaaaaaaaaaaaaaaaaaaaaaaaa

SEQ ID NO: 38-44 - skipped (7 entries)

SEQ ID NO: 45 - DNA, 28 bp, Artificial Sequence
  Synthetic Oligonucleotide
caugcgcuuuucugagaagcaacgcaug

SEQ ID NO: 46 - DNA, 30 bp, Artificial Sequence
  Synthetic Oligonucleotide
cugagaagcaacuucucuauuaacgcucag

SEQ ID NO: 47 - skipped

SEQ ID NO: 48 - DNA, 59 bp, Artificial Sequence
  Synthetic Oligonucleotide
  misc_feature (27)..(59): 3' Tail
gctcagaaaaccagaagcgaaacgggtttaaaaaaaaaaaaaaaaaaaaaaaaaaaaaa

SEQ ID NO: 49-59 - skipped (11 entries)

SEQ ID NO: 60 - DNA, 22 bp, Artificial Sequence
  Synthetic Oligonucleotide
ggaugugacugucaugccaucc

SEQ ID NO: 61-63 - skipped (3 entries)

SEQ ID NO: 64 - DNA, 26 bp, Artificial Sequence
  Synthetic Oligonucleotide
gaauggcgccguggaugguugcauuc

SEQ ID NO: 65 - DNA, 53 bp, Artificial Sequence
  Synthetic Oligonucleotide
  misc_feature (21)..(53): 3' Tail
agaucgguaucgggugcuugtttaaaaaaaaaaaaaaaaaaaaaaaaaaaaaa

SEQ ID NO: 66 - DNA, 50 bp, Artificial Sequence
  Synthetic Oligonucleotide
  misc_feature (18)..(50): 3' Tail
gatggagcgtaccaccgtttaaaaaaaaaaaaaaaaaaaaaaaaaaaaaa

SEQ ID NO: 67 - DNA, 49 bp, Artificial Sequence
  Synthetic Oligonucleotide
  misc_feature (17)..(49): 3' Tail
cggtatcgggtgcttgtttaaaaaaaaaaaaaaaaaaaaaaaaaaaaaa

SEQ ID NO: 68 - skipped

SEQ ID NO: 69 - DNA, 49 bp, Artificial Sequence
  Synthetic Oligonucleotide
  misc_feature (17)..(49): 3' Tail
ccagaagcgaaacgggtttaaaaaaaaaaaaaaaaaaaaaaaaaaaaaa

SEQ ID NO: 70-71 - skipped (2 entries)

SEQ ID NO: 72 - DNA, 20 bp, Artificial Sequence
  Synthetic Oligonucleotide
gctgtaaaaggcttacttcg

SEQ ID NO: 73 - DNA, 21 bp, Artificial Sequence
  Synthetic Oligonucleotide
cttccttagcgtgaaaacgca

SEQ ID NO: 74 - DNA, 23 bp, Artificial Sequence
  Synthetic Oligonucleotide
aggctgtaaaaggtctgcttcgt

SEQ ID NO: 75 - DNA, 19 bp, Artificial Sequence
  Synthetic Oligonucleotide
agaaatcttcagagcccga

SEQ ID NO: 76 - skipped

SEQ ID NO: 77 - DNA, 19 bp, Artificial Sequence
  Synthetic Oligonucleotide
tcaagttcgcatattgcac

SEQ ID NO: 78 - skipped

SEQ ID NO: 79 - DNA, 18 bp, Artificial Sequence
  Synthetic Oligonucleotide
accgacatccttacgtag

SEQ ID NO: 80 - DNA, 22 bp, Artificial Sequence
  Synthetic Oligonucleotide
atactggaccgacatccttacg

SEQ ID NO: 81-83 - skipped (3 entries)

SEQ ID NO: 84 - DNA, 20 bp, Artificial Sequence
  Synthetic Oligonucleotide
agatcggtatcgggtgcttg

SEQ ID NO: 85-86 - skipped (2 entries)

SEQ ID NO: 87 - DNA, 26 bp, Artificial Sequence
  Synthetic Oligonucleotide
gctcagaaaaccagaagcgaaacggg

SEQ ID NO: 88 - skipped

SEQ ID NO: 89 - DNA, 20 bp, Artificial Sequence
  Synthetic Oligonucleotide
agaucgguaucgggugcuug

SEQ ID NO: 90 - DNA, 17 bp, Artificial Sequence
  Synthetic Oligonucleotide
gatggagcgtaccaccg

SEQ ID NO: 91 - DNA, 16 bp, Artificial Sequence
  Synthetic Oligonucleotide
cggtatcgggtgcttg

SEQ ID NO: 92 - skipped

SEQ ID NO: 93 - DNA, 16 bp, Artificial Sequence
  Synthetic Oligonucleotide
ccagaagcgaaacggg

SEQ ID NO: 94-97 - skipped (4 entries)

SEQ ID NO: 98 - DNA, 19 bp, Artificial Sequence
  Synthetic Oligonucleotide
tcggtatcgggtgcttgaa

SEQ ID NO: 99 - DNA, 25 bp, Artificial Sequence
  Synthetic Oligonucleotide
ggatggagcgtaccaccgaatttcc

SEQ ID NO: 100 - DNA, 20 bp, Artificial Sequence
  Synthetic Oligonucleotide
taccaccgaatttcccaccc

SEQ ID NO: 101 - skipped

SEQ ID NO: 102 - DNA, 20 bp, Artificial Sequence
  Synthetic Oligonucleotide
ccaaguccuuguggcuuggc

SEQ ID NO: 103-105 - skipped (3 entries)

SEQ ID NO: 106 - DNA, 17 bp, Artificial Sequence
  Synthetic Oligonucleotide
gguggauuugugcgaca

SEQ ID NO: 107 - DNA, 22 bp, Artificial Sequence
  Synthetic Oligonucleotide
augggaauggcgccguggaugg

SEQ ID NO: 108 - DNA, 20 bp, Artificial Sequence
  Synthetic Oligonucleotide
ggcagagacguaugggccug

SEQ ID NO: 109 - DNA, 22 bp, Artificial Sequence
  Synthetic Oligonucleotide
ggaauggcgccguggaugguug

SEQ ID NO: 110 - DNA, 18 bp, Artificial Sequence
  Synthetic Oligonucleotide
cagccaaccauccacggc

SEQ ID NO: 111-112 - skipped (2 entries)

SEQ ID NO: 113 - DNA, 23 bp, Artificial Sequence
  Synthetic Oligonucleotide
caugcgcuuuucugagaagcaac

SEQ ID NO: 114 - DNA, 25 bp, Artificial Sequence
  Synthetic Oligonucleotide
cugagaagcaacuucucuauuaacg

SEQ ID NO: 115-123 - skipped (9 entries)

SEQ ID NO: 124 - DNA, 17 bp, Artificial Sequence
  Synthetic Oligonucleotide
ggaugugacugucaugc

SEQ ID NO: 125-127 - skipped (3 entries)

SEQ ID NO: 128 - DNA, 21 bp, Artificial Sequence
  Synthetic Oligonucleotide
gaauggcgccguggaugguug

SEQ ID NO: 129 - DNA, 308 bp, Candida albicans
  ref <308>: DQ660433.1
  ref <309>: 2007-03-10
  ref <313>: (1)..(308)
ccggtcaacataaggagttttctttagaaactcattcacaaccaaatgcgggtgggaaattcggtggtacgctccatcctttacagatttgctcctgagagcttcttccttagcgtgaaagcgcatgggcggcgttacaagaaatatacacggagttttaaggctgtagaaggtctgcttcgtatgggaatggcgccgtggatggttggctgtgagtaattctttactacaagctgtttagtgcaatatgcgaacttgaagtcaccttcaagcacccgataccgatcaccgacttgagacaggtttta

SEQ ID NO: 130 - DNA, 365 bp, Candida parapsilosis
  ref <308>: DQ660436.1
  ref <309>: 2007-03-10
  ref <313>: (1)..(365)
gagctcgactcgtctcgattcgcattgacccgcgaacaaaaggaactttccgttcaaaagcaaaaattatgcgggtgggaaattcggtggtactctccattcattcaagatttgtgctcctgagagcaaattcctgagcgtgcaaacgcatgggcggtgttaaaagaaatcttcagagcccgaaggcgcccgactaccttcggtagtttggcttttctttgggttctatgggaatgacgccgtgaatggttggctgttgtttagtgtcaaagcgaacaagggctatttagtgcaatatgcgaacttgatggttgttcataactgtcaagaacccgataccgatcattgacgatgagttgagttaa

SEQ ID NO: 131 - DNA, 1008 bp, Candida glabrata
  ref <308>: DQ660434.2
  ref <309>: 2007-03-21
  ref <313>: (1)..(1008)
ggattacagcttagtggagcttggagtataggtgctcctctgagttcattttgagcctctgggtactcttgagagtactgactcttacgcggttggttacatgtggtttgaaggtcttttctgagggtttttctgttggaggttacgggagttgtgtgtgtcggtgtattgtcgtggagcttcacttggagttgtctgcgtctcagagcaagtcgtggggattatgtcttttggctgtccgttcgttttcctcttcacctttctgcttgtacaataggtcttgtagagctccagtgctattcttagtcgaccgtgaggacggctttcgggggaacccggccggtaagattaagtgcattggagtttctgctgaaatctgtatcgtataaggaggataagggtggggcagagacgtatgggcctgtctagggatgtgactgtcatgcgcttttctgagaagcaacttctctattaacggtggatttgtgcgacacttctccattgctcacttcctctctaatggagggccctacgtaaggatgtcggtccagtatgtctgcgattgtttctgtggtggacctcgcgctgttataagaaatatacccgtttcgcttctggttttctgagcaggaagatatatttccagtgaagatgcaccaggagcaacggctgggaatggcagcggattaagaaagccactgaaaactctcgcaggtgcattgggtagagaaagcctgcgtattttctttccacatattcctacatcactatgaagggtggagctttcctctcttcagagatgttccgtagttctctggggtgcttagtttgatcatgtggtgcgtcttcttcttagtttcacggcttggctcacacactttgtcgctttaaacctgccatttccgctctcttaagagagtgcattggtgtgaggcgaggtgtcaaaatcgtggtgaggctttattcagtgcaattgtaggacttgtcgtctcgttagagatgatttga

SEQ ID NO: 132 - DNA, 25 bp, Artificial Sequence
  Synthetic Oligonucleotide
gcggcgttacaagaaatatacacgg

SEQ ID NO: 133 - DNA, 14 bp, Artificial Sequence
  Synthetic Oligonucleotide
gttacaagaaatat

SEQ ID NO: 134 - DNA, 25 bp, Artificial Sequence
  Synthetic Oligonucleotide
atactggaccgacatccttacgtag

SEQ ID NO: 135 - DNA, 15 bp, Artificial Sequence
  Synthetic Oligonucleotide
accgacatccttacg

SEQ ID NO: 136 - DNA, 21 bp, Artificial Sequence
  Synthetic Oligonucleotide
agtgcattggagtttctgctg

SEQ ID NO: 137 - DNA, 16 bp, Artificial Sequence
  Synthetic Oligonucleotide
gcattggagtttctgc

SEQ ID NO: 138 - DNA, 22 bp, Artificial Sequence
  Synthetic Oligonucleotide
agatcggtatcgggtgcttgaa

SEQ ID NO: 139 - DNA, 16 bp, Artificial Sequence
  Synthetic Oligonucleotide
cggtatcgggtgcttg

SEQ ID NO: 140 - DNA, 30 bp, Artificial Sequence
  Synthetic Oligonucleotide
ggatggagcgtaccaccgaatttcccaccc

SEQ ID NO: 141 - skipped

SEQ ID NO: 142 - DNA, 42 bp, Artificial Sequence
  Synthetic Oligonucleotide
ggaaatatatcttcctgctcagaaaaccagaagcgaaacggg

SEQ ID NO: 143 - DNA, 16 bp, Artificial Sequence
  Synthetic Oligonucleotide
ccagaagcgaaacggg

SEQ ID NO: 144 - skipped

SEQ ID NO: 145 - DNA, 29 bp, Artificial Sequence
  Synthetic Oligonucleotide
augggaauggcgccguggaugguuggcug

SEQ ID NO: 146 - DNA, 14 bp, Artificial Sequence
  Synthetic Oligonucleotide
gccguggaugguug

SEQ ID NO: 147 - DNA, 35 bp, Artificial Sequence
  Synthetic Oligonucleotide
ggaugugacugucaugcgcuuuucugagaagcaac

SEQ ID NO: 148 - skipped

SEQ ID NO: 149 - DNA, 23 bp, Artificial Sequence
  Synthetic Oligonucleotide
gccguggaugguuggcugacggc

SEQ ID NO: 150 - DNA, 18 bp, Artificial Sequence
  Synthetic Oligonucleotide
gccguggaugguuggcug

SEQ ID NO: 151 - DNA, 20 bp, Artificial Sequence
  Synthetic Oligonucleotide
gctgtaaaaggyytrcttcg

SEQ ID NO: 152 - DNA, 23 bp, Artificial Sequence
  Synthetic Oligonucleotide
aggctgtaaaaggyytrcttcgt

SEQ ID NO: 153 - DNA, 16 bp, Artificial Sequence
  Synthetic Oligonucleotide
gtgaaagcgcatgggc

SEQ ID NO: 154 - DNA, 21 bp, Artificial Sequence
  Synthetic Oligonucleotide
gaaatcttcagagcccgaagg

SEQ ID NO: 155 - DNA, 28 bp, Artificial Sequence
  Synthetic Oligonucleotide
ggaauggcgccguggaugguugcauucc